European Patent Specification EP 3 259 370 B1, published January 8, 2025. Title: Method of DNA synthesis. Applicant: Touchlight Genetics Limited. The sequence listing filed with the application follows.

SEQUENCE LISTING (43 sequences)

SEQ ID NO: 1 - DNA, 1563 bp, Halomonas aquamarina phage phiHAP-1
  misc_feature: Protelomerase
atgagcggtgagtcacgtagaaaggtcgatttagcggaattgatagagtggttgctcagcgagatcaaagagatcgacgccgatgatgagatgccacgtaaagagaaaaccaagcgcatggcgcggctggcacgtagcttcaaaacgcgcctgcatgatgacaagcgccgcaaggattctgagcggatcgcggtcacgacctttcgccgctacatgacagaagcgcgcaaggcggtgactgcgcagaactggcgccatcacagcttcgaccagcagatcgagcggctggccagccgctacccggcttatgccagcaagctggaagcgctcggcaagctgaccgatatcagcgccattcgtatggcccaccgcgagctgctcgaccagatccgcaacgatgacgacgcttatgaggacatccgggcgatgaagctggaccatgaaatcatgcgccacctgacgttgagctctgcacagaaaagcacgctggctgaagaggccagcgagacgctggaagagcgcgcggtgaacacggtcgagatcaactaccactggttgatggagacggtttacgagctgctgagtaaccgggagagaatggtcgatggggagtatcgcggctttttcagttacctagcgcttgggctggcgctggccaccgggcgtcgctcgatcgaggtgctgaagaccggacggatcacgaaggtgggcgagtatgagctggagttcagcggccaggcgaaaaagcgcggcggcgtcgactatagcgaggcttaccacatttataccctggtgaaagctgacctggtgatcgaagcgtgggatgagcttcgctcgctgccggaagctgctgagctgcagggcatggacaacagcgatgtgaaccgccgcacggcgaagacgctcaacacgctcactaagcggatctttaacaacgatgagcgcgttttcaaggacagccgggcgatctgggcgcggctggtgtttgagctgcacttctcgcgcgacaagcgctggaagaaagtcaccgaggacgtgttctggcgtgagatgctggggcatgaggacatggatacacagcgcagctaccgcgcctttaaaatcgactacgacgagccggatcaagccgaccaggaagattacgaacacgctagccgcctcgccgcgctgcaggcgctggacggccatgagcagcttgagagcagcgacgcccaggcgcgtgtgcatgcctgggtgaaagcgcagatcgagcaggagcctgacgcgaaaattacgcagtctctgatcagccgggagctgggcgtttatcgccctgccataaaagcgtacctggagctggcgcgagaggcgctcgacgcgccgaacgtcgatctggacaaggtcgcggcggcagtgccgaaggaagtagccgaggcgaagccccggctgaacgcccacccacaaggggatggcaggtgggtcggggtggcttcaatcaacggggtggaagttgcacgggtgggcaaccaggcaggccggatcgaagcgatgaaagcggcctataaagcggcgggtgggcgctga

SEQ ID NO: 2 - protein, 520 aa, Halomonas aquamarina phage phiHAP-1
  MISC_FEATURE: Protelomerase
MSGESRRKVDLAELIEWLLSEIKEIDADDEMPRKEKTKRMARLARSFKTRLHDDKRRKDSERIAVTTFRRYMTEARKAVTAQNWRHHSFDQQIERLASRYPAYASKLEALGKLTDISAIRMAHRELLDQIRNDDDAYEDIRAMKLDHEIMRHLTLSSAQKSTLAEEASETLEERAVNTVEINYHWLMETVYELLSNRERMVDGEYRGFFSYLALGLALATGRRSIEVLKTGRITKVGEYELEFSGQAKKRGGVDYSEAYHIYTLVKADLVIEAWDELRSLPEAAELQGMDNSDVNRRTAKTLNTLTKRIFNNDERVFKDSRAIWARLVFELHFSRDKRWKKVTEDVFWREMLGHEDMDTQRSYRAFKIDYDEPDQADQEDYEHASRLAALQALDGHEQLESSDAQARVHAWVKAQIEQEPDAKITQSLISRELGVYRPAIKAYLELAREALDAPNVDLDKVAAAVPKEVAEAKPRLNAHPQGDGRWVGVASINGVEVARVGNQAGRIEAMKAAYKAAGGR

SEQ ID NO: 3 - DNA, 1854 bp, Yersinia enterolytica phage PY54
  misc_feature: Protelomerase
atgaaaatccattttcgcgatttagttagtggtttagttaaagagatcgatgaaatagaaaaatcagaccgggcgcagggtgacaaaactcggcgttatcagggcgcggccagaaagttcaaaaatgccgtgtttatggataaacggaaatatcgcggtaacggtatgaagaatagaatatcgttaacaacatttaataaatatttaagtcgagcacgttctcggtttgaagaaaggcttcaccatagttttcctcaatctatagcaactatctcaaataaatatcctgcattcagcgaaataataaaagatctggataatagacccgctcatgaagttagaataaaacttaaagaattaataactcatcttgaatccggtgttaatttattagaaaaaataggtagcttagggaaaataaaaccatctacagctaaaaaaatagttagcttaaaaaaaatgtacccatcatgggctaatgatctagatactttaattagtactgaagatgctacagaattacaacaaaagttagagcaagggaccgacctacttaacgcattacattctctaaaagtaaaccatgaagttatgtatgcattaacgatgcagccttctgacagagctgcattaaaagctaggcatgacgctgcccttcactttaaaaagcgtaacatcgtacctatcgattatcccggctatatgcaacgaatgacggacatactacatcttccagatatagcttttgaagattcgatggcatcacttgcccctttagcatttgctctagcagctgctagcggtcgcagacaaattgaaatactaattactggtgagtttgacgccaaaaataaaagcatcattaaattttctggacaagcaaaaaaaagaatggccgtttcaggtggacattatgaaatatacagtctaattgactcagagctattcattcaacggttagagtttttacgttctcatagctcaatacttcgattacaaaatttggaaatagcacatgatgaacatcgtactgaactatctgttattaacggttttgtagccaaacctttaaatgatgcagcaaaacagttctttgtcgatgacagaagagtatttaaagatacccgtgcaatttacgctcgcatagcatatgaaaaatggtttagaacagatcctcgctgggcgaagtgcgacgaagatgttttcttctctgaattattaggccatgacgacccagatactcagctggcatataaacaattcaagctggtaaatttcaatccaaaatggacacctaatatatcagatgaaaaccctcggttagctgcacttcaagagcttgacaatgatatgcccggcctagcacgtggcgatgcggcagttcgcatacatgagtgggttaaagagcaactggcgcagaaccctgcggcaaaaataactgcataccaaatcaagaaaaatttaaattgtcgaaatgacttggccagccgatacatggcatggtgtgctgacgcgctaggggttgttattggtgatgatggacaggcaaggccagaagaactcccaccatcgctcgtgcttgatattaacgctgatgacactgacgctgaagaagatgaaatagaggaagactttactgatgaggaaatagacgacaccgaattcgacgtatcagataacgccagtgatgaagataagcccgaagataaacctcgctttgcagcaccaattcgtagaagtgaggactcttggctgattaaatttgaatttgctggcaagcaatatagctgggagggtaatgccgaaagtgttatcgatgcgatgaaacaagcatggactgaaaatatggagtaa

SEQ ID NO: 4 - protein, 617 aa, Yersinia enterolytica phage PY54
  MISC_FEATURE: Protelomerase
MKIHFRDLVSGLVKEIDEIEKSDRAQGDKTRRYQGAARKFKNAVFMDKRKYRGNGMKNRISLTTFNKYLSRARSRFEERLHHSFPQSIATISNKYPAFSEIIKDLDNRPAHEVRIKLKELITHLESGVNLLEKIGSLGKIKPSTAKKIVSLKKMYPSWANDLDTLISTEDATELQQKLEQGTDLLNALHSLKVNHEVMYALTMQPSDRAALKARHDAALHFKKRNIVPIDYPGYMQRMTDILHLPDIAFEDSMASLAPLAFALAAASGRRQIEILITGEFDAKNKSIIKFSGQAKKRMAVSGGHYEIYSLIDSELFIQRLEFLRSHSSILRLQNLEIAHDEHRTELSVINGFVAKPLNDAAKQFFVDDRRVFKDTRAIYARIAYEKWFRTDPRWAKCDEDVFFSELLGHDDPDTQLAYKQFKLVNFNPKWTPNISDENPRLAALQELDNDMPGLARGDAAVRIHEWVKEQLAQNPAAKITAYQIKKNLNCRNDLASRYMAWCADALGVVIGDDGQARPEELPPSLVLDINADDTDAEEDEIEEDFTDEEIDDTEFDVSDNASDEDKPEDKPRFAAPIRRSEDSWLIKFEFAGKQYSWEGNAESVIDAMKQAWTENME

SEQ ID NO: 5 - DNA, 1923 bp, Klebsiella phage phiKO2
  misc_feature: Protelomerase
atgcgtaaggtgaaaattggtgagctaatcaattcgcttgtgagcgaggtcgaggcaatcgatgcctctgatcgtccgcaaggcgataaaacgaagaaaattaaagccgcagcattaaaatataagaatgcattatttaatgacaaaagaaagtttcgcggtaaaggtttagaaaaaagaatttctgccaacacgttcaactcgtatatgagtcgggcaaggaaaagatttgatgatagattgcatcataactttgaaaagaatgtaattaaactatcagaaaaatatcctttatatagtgaagaattatcttcgtggctttctatgcctgcggcatcaattagacagcatatgtcaagattgcaagccaagctaaaagagataatgccattggcagaagacttatccaatataaagattggtacaaaaaatagcgaagcaaaaataaataaactcgctaataaatatcctgaatggcaattcgctattagtgatttaaatagcgaagattggaaggataaaagagattatctttataaactattccaacaaggttcttcgctcctggaagacttgaataacctgaaagtaaaccatgaggttctctatcatctgcagcttagttctgccgagcgaacctctatccagcagcgctgggccaacgtcctcagcgagaaaaagcgcaacgttgtcgtgattgactatccgcgctatatgcaggccatctacgatataatcaacaagcctatagtttcgttcgatttgactactcgtcgtggtatggccccgctggcgttcgcccttgccgcgctatctggtcgccgaatgattgaaatcatgctccagggtgaattttccgtcgcaggtaaatatacagtaacattcctggggcaagctaaaaaacgctcggaagataaaggtatatcaaggaaaatatataccttatgcgacgctactttatttgttagtttggtaaatgaacttcgctcatgccccgctgctgcggattttgatgaagtaataaaaggatatggcgaaaatgacactcgctcagaaaatgggcgtattaatgcaattctcgctacagcttttaatccgtgggtaaaaactttcttaggcgatgaccgccgcgtttataaagatagccgcgctatttacgcccgtattgcctatgaaatgttcttccgcgttgaccctcggtggaagaatgttgatgaggatgtattcttcatggagattctcggccatgacgatgaaaacacccaactgcactataagcagtttaaattggctaacttctccagaacatggcgaccaaatgtcggcgaggagaatgcccgcctagcggcgctgcaaaagctggatagcatgatgccagattttgccaggggcgacgccggggttcgtattcatgagaccgtgaagcagctggtggagcaggacccatcgataaaaatcacaaacagcaccctgcgaccgtttaacttcagtaccaggctgattcctcgctacctggagtttgccgccgatgcattgggccagttcgtcggtgaaaatgggcaatggcaactgaaggatgaggcgcctgcaatagtcctgcctgatgaggaaattcttgagcctatggacgacgtcgatctcgatgacgaaaaccatgatgatgaaacgctggatgacgatgagatcgaagtggacgaaagcgaaggagaggaactggaggaagcgggcgacgctgaagaggccgaggtggctgaacaggaagagaagcaccctggcaagccaaactttaaagcgccgagggataatggcgatggtacctacatggtggaatttgaattcggtggccgtcattacgcctggtccggtgccgccggtaatcgggtagaggcaatgcaatctgcctggagtgcctacttcaagtga

SEQ ID NO: 6 - protein, 640 aa, Klebsiella phage phiKO2
  MISC_FEATURE: Protelomerase
MRKVKIGELINSLVSEVEAIDASDRPQGDKTKKIKAAALKYKNALFNDKRKFRGKGLEKRISANTFNSYMSRARKRFDDRLHHNFEKNVIKLSEKYPLYSEELSSWLSMPAASIRQHMSRLQAKLKEIMPLAEDLSNIKIGTKNSEAKINKLANKYPEWQFAISDLNSEDWKDKRDYLYKLFQQGSSLLEDLNNLKVNHEVLYHLQLSSAERTSIQQRWANVLSEKKRNVVVIDYPRYMQAIYDIINKPIVSFDLTTRRGMAPLAFALAALSGRRMIEIMLQGEFSVAGKYTVTFLGQAKKRSEDKGISRKIYTLCDATLFVSLVNELRSCPAAADFDEVIKGYGENDTRSENGRINAILATAFNPWVKTFLGDDRRVYKDSRAIYARIAYEMFFRVDPRWKNVDEDVFFMEILGHDDENTQLHYKQFKLANFSRTWRPNVGEENARLAALQKLDSMMPDFARGDAGVRIHETVKQLVEQDPSIKITNSTLRPFNFSTRLIPRYLEFAADALGQFVGENGQWQLKDEAPAIVLPDEEILEPMDDVDLDDENHDDETLDDDEIEVDESEGEELEEAGDAEEAEVAEQEEKHPGKPNFKAPRDNGDGTYMVEFEFGGRHYAWSGAAGNRVEAMQSAWSAYFK

SEQ ID NO: 7 - DNA, 1617 bp, Vibrio sp. phage VP882
  misc_feature: Protelomerase
atgagcggcgaaagtagacaaaaggtaaacctcgaggagttaataaatgagctcgtcgaggaggtgaaaaccatcgatgacaatgaggcgattactcggtctgaaaaaaccaagttgatcaccagggcggcgactaaattcaagaccaagctgcacgacgataagcgccggaaggatgcgaccagaatcgctctgagcacctatcgtaagtacatgacaatggccagggcagcagttactgagcagaactggaaacaccacagtctcgagcagcagatagagcggctggccaaaaagcacccgcaatacgctgagcagctggtggccatcggggccatggataacatcaccgagttgcgcctggcgcatcgcgacctcctgaagagcatcaaggacaacgatgaagccttcgaggatatccgcagcatgaagttagaccacgaggtaatgcgccatctgacgctacccagtgcgcaaaaggcgagactggcagaggaagccgccgaggcgttgaccgagaagaaaaccgccacggtcgacatcaactatcacgagctgatggccggcgtggtggagctgttgaccaagaagaccaagacggtcggcagcgacagcacctacagcttcagccggctggcgcttggtattggcctggctaccggtcgtcgttctatcgagatactgaagcagggcgagttcaaaaaggtggatgagcagcggctcgagttctctggccaagcgaaaaagcgcggcggtgccgactattcagagacctataccatttacaccctggtcgactccgacctggtactgatggcgctgaagaacctgcgagagttgccagaagttcgcgcactggatgagtacgaccaactgggcgagattaagcggaacgacgccatcaataaacgctgtgcaaaaacgctcaaccaaaccgccaagcagttctttggcagcgacgagcgcgtgttcaaagatagtcgtgccatctgggcgcgtctggcttatgagttgttttttcaacgtgatccgcgctggaaaaagaaagacgaggacgttttctggcaggagatgctgggccacgaggacatcgagactcagaaagcctataagcaattcaaggtcgactacagcgaacctgagcagccggtgcacaagcctggcaaatttaagagcagagctgaagccctcgcggcgctcgactcaaatgaggacattaccacccgctcatccatggccaagatccacgactgggtgaaagagcgtattgcggaagaccccgaggcgaacatcacacagtcactcatcacccgggaactgggctcaggccgtaaggtgatcaaggactacctcgacctggctgacgatgcccttgctgtggtgaatactcctgtcgatgacgcagtcgtcgaggttccagctgatgtgccggcagcagaaaaacagccgaagaaagcgcagaagcccagactcgtggctcaccaggttgatgatgagcactgggaagcctgggcgctggtggaaggcgaggaggtggccagggtgaaaatcaagggcacccgcgttgaggcaatgacagccgcatgggaggccagccaaaaggcactcgatgactaa

SEQ ID NO: 8 - protein, 538 aa, Vibrio sp. phage VP882
  MISC_FEATURE: Protelomerase
MSGESRQKVNLEELINELVEEVKTIDDNEAITRSEKTKLITRAATKFKTKLHDDKRRKDATRIALSTYRKYMTMARAAVTEQNWKHHSLEQQIERLAKKHPQYAEQLVAIGAMDNITELRLAHRDLLKSIKDNDEAFEDIRSMKLDHEVMRHLTLPSAQKARLAEEAAEALTEKKTATVDINYHELMAGVVELLTKKTKTVGSDSTYSFSRLALGIGLATGRRSIEILKQGEFKKVDEQRLEFSGQAKKRGGADYSETYTIYTLVDSDLVLMALKNLRELPEVRALDEYDQLGEIKRNDAINKRCAKTLNQTAKQFFGSDERVFKDSRAIWARLAYELFFQRDPRWKKKDEDVFWQEMLGHEDIETQKAYKQFKVDYSEPEQPVHKPGKFKSRAEALAALDSNEDITTRSSMAKIHDWVKERIAEDPEANITQSLITRELGSGRKVIKDYLDLADDALAVVNTPVDDAVVEVPADVPAAEKQPKKAQKPRLVAHQVDDEHWEAWALVEGEEVARVKIKGTRVEAMTAAWEASQKALDD

SEQ ID NO: 9 - DNA, 4055 bp, Escherichia coli bacteriophage N15
  misc_feature: Protelomerase TelN
catatgcactatatcatatctcaattacggaacatatcagcacacaattgcccattatacgcgcgtataatggactattgtgtgctgataaggagaacataagcgcagaacaatatgtatctattccggtgttgtgttcctttgttattctgctattatgttctcttatagtgtgacgaaagcagcataattaatcgtcacttgttctttgattgtgttacgatatccagagacttagaaacgggggaaccgggatgagcaaggtaaaaatcggtgagttgatcaacacgcttgtgaatgaggtagaggcaattgatgcctcagaccgcccacaaggcgacaaaacgaagagaattaaagccgcagccgcacggtataagaacgcgttatttaatgataaaagaaagttccgtgggaaaggattgcagaaaagaataaccgcgaatacttttaacgcctatatgagcagggcaagaaagcggtttgatgataaattacatcatagctttgataaaaatattaataaattatcggaaaagtatcctctttacagcgaagaattatcttcatggctttctatgcctacggctaatattcgccagcacatgtcatcgttacaatctaaattgaaagaaataatgccgcttgccgaagagttatcaaatgtaagaataggctctaaaggcagtgatgcaaaaatagcaagactaataaaaaaatatccagattggagttttgctcttagtgatttaaacagtgatgattggaaggagcgccgtgactatctttataagttattccaacaaggctctgcgttgttagaagaactacaccagctcaaggtcaaccatgaggttctgtaccatctgcagctaagccctgcggagcgtacatctatacagcaacgatgggccgatgttctgcgcgagaagaagcgtaatgttgtggttattgactacccaacatacatgcagtctatctatgatattttgaataatcctgcgactttatttagtttaaacactcgttctggaatggcacctttggcctttgctctggctgcggtatcagggcgaagaatgattgagataatgtttcagggtgaatttgccgtttcaggaaagtatacggttaatttctcagggcaagctaaaaaacgctctgaagataaaagcgtaaccagaacgatttatactttatgcgaagcaaaattattcgttgaattattaacagaattgcgttcttgctctgctgcatctgatttcgatgaggttgttaaaggatatggaaaggatgatacaaggtctgagaacggcaggataaatgctattttagcaaaagcatttaacccttgggttaaatcatttttcggcgatgaccgtcgtgtttataaagatagccgcgctatttacgctcgcatcgcttatgagatgttcttccgcgtcgatccacggtggaaaaacgtcgacgaggatgtgttcttcatggagattctcggacacgacgatgagaacacccagctgcactataagcagttcaagctggccaacttctccagaacctggcgacctgaagttggggatgaaaacaccaggctggtggctctgcagaaactggacgatgaaatgccaggctttgccagaggtgacgctggcgtccgtctccatgaaaccgttaagcagctggtggagcaggacccatcagcaaaaataaccaacagcactctccgggcctttaaatttagcccgacgatgattagccggtacctggagtttgccgctgatgcattggggcagttcgttggcgagaacgggcagtggcagctgaagatagagacacctgcaatcgtcctgcctgatgaagaatccgttgagaccatcgacgaaccggatgatgagtcccaagacgacgagctggatgaagatgaaattgagctcgacgagggtggcggcgatgaaccaaccgaagaggaagggccagaagaacatcagccaactgctctaaaacccgtcttcaagcctgcaaaaaataacggggacggaacgtacaagatagagtttgaatacgatggaaagcattatgcctggtccggccccgccgatagccctatggccgcaatgcgatccgcatgggaaacgtactacagctaaaagaaaagccaccggtgttaatcggtggcttttttattgaggcctgtccctacccatcccctgcaagggacggaaggattaggcggaaactgcagctgcaactacggacatcgccgtcccgactgcagggacttccccgcgtaaagcggggcttaaattcgggctggccaaccctatttttctgcaatcgctggcgatgttagtttcgtggatagcgtttccagcttttcaatggccagctcaaaatgtgctggcagcaccttctccagttccgtatcaatatcggtgatcggcagctctccacaagacatactccggcgaccgccacgaactacatcgcgcagcagctcccgttcgtagacacgcatgttgcccagagccgtttctgcagccgttaatatccggcgcacgtcggcgatgattgccgggagatcatccacggttattgggttcggtgatgggttcctgcaggcgcggcggagagccatccagacgccgctaacccatgcgttacggtactgaaaactttgtgctatgtcgtttatcaggcccgaagttcttctttctgccgccagtccagtggttcaccggcgttcttaggctcaggctcgacaaaagcatactcgccgtttttccggatagctggcagaacctcgttcgtcacccacttgcggaaccgccaggctgtcgtcccctgtttcaccgcgtcgcggcagcggaggattatggtgtagagaccagattccgataccacatttacttccctggccatccgatcaagtttttgtgcctcggttaaaccgagggtcaatttttcatcatgatccagcttacgcaatgcatcagaagggttggctatattcaatgcagcacagatatccagcgccacaaaccacgggtcaccaccgacaagaaccacccgtatagggtggctttcctgaaatgaaaagacggagagagccttcattgcgcctccccggatttcagctgctcagaaagggacagggagcagccgcgagcttcctgcgtgagttcgcgcgcgacctgcagaagttccgcagcttcctgcaaatacagcgtggcctcataactggagatagtgcggtgagcagagcccacaagcgcttcaacctgcagcaggcgttcctcaatcgtctccagcaggccctgggcgtttaactgaatctggttcatgcgatcacctcgctgaccgggatacgggctgacagaacgaggacaaaacggctggcgaactggcgacgagcttctcgctcggatgatgcaatggtggaaaggcggtggatatgggattttttgtccgtgcggacgacagctgcaaatttgaatttgaacatggtatgcattcctatcttgtatagggtgctaccaccagagttgagaatctctataggggtggtagcccagacagggttctcaacaccggtacaagaagaaaccggcccaaccgaagttggccccatctgagccaccataattcaggtatgcgcagatttaacacacaaaaaaacacgctggcgcgtgttgtgcgcttcttgtcattcggggttgagaggcccggctgcagattttgctgcagcggggtaactctaccgccaaagcagaacgcacgtcaataatttaggtggatattttaccccgtgaccagtcacgtgcacaggtgtttttatagtttgctttactgactgatcagaacctgatcagttattggagtccggtaatcttattgatgaccgcagccaccttagatgttgtctcaaaccccatacggccacgaatgagccactggaacggaatagtcagcaggtacagcggaacgaaccacaaacggttcagacgctgccagaacgtcgcatcacgacgttccatccattcggtattgtcgac

SEQ ID NO: 10 - protein, 631 aa, Escherichia coli bacteriophage N15
  misc_feature: Protelomerase sequence Tel N
MSKVKIGELINTLVNEVEAIDASDRPQGDKTKRIKAAAARYKNALFNDKRKFRGKGLQKRITANTFNAYMSRARKRFDDKLHHSFDKNINKLSEKYPLYSEELSSWLSMPTANIRQHMSSLQSKLKEIMPLAEELSNVRIGSKGSDAKIARLIKKYPDWSFALSDLNSDDWKERRDYLYKLFQQGSALLEELHQLKVNHEVLYHLQLSPAERTSIQQRWADVLREKKRNVVVIDYPTYMQSIYDILNNPATLFSLNTRSGMAPLAFALAAVSGRRMIEIMFQGEFAVSGKYTVNFSGQAKKRSEDKSVTRTIYTLCEAKLFVELLTELRSCSAASDFDEVVKGYGKDDTRSENGRINAILAKAFNPWVKSFFGDDRRVYKDSRAIYARIAYEMFFRVDPRWKNVDEDVFFMEILGHDDENTQLHYKQFKLANFSRTWRPEVGDENTRLVALQKLDDEMPGFARGDAGVRLHETVKQLVEQDPSAKITNSTLRAFKFSPTMISRYLEFAADALGQFVGENGQWQLKIETPAIVLPDEESVETIDEPDDESQDDELDEDEIELDEGGGDEPTEEEGPEEHQPTALKPVFKPAKNNGDGTYKIEFEYDGKHYAWSGPADSPMAAMRSAWETYYS

SEQ ID NO: 11 - DNA, 1329 bp, Agrobacterium tumefaciens strain C58
  misc_feature: Protelomerase TelA
atgctcgccgcaaaacgaaaaacaaaaacaccggtcctcgtggaacgcatcgatcaattcgtcggccagatcaaagaggcgatgaaaagcgacgacgcttcgcgaaacaggaaaatccgcgatctgtgggatgccgaggtccgctatcatttcgataatggccgcacggaaaagacgctcgaactttacatcatgaaatatcgcaatgcgctgaaggccgaattcggcccgaagagcaccccgctagccatctgcaacatgaagaagctgcgcgagcgcctgaacacctatattgcccggggcgattatcccaagacaggcgtggcgacgtcgattgtcgaaaaaatcgagcgggcggagttcaacaccgccggccgcaaacccacggttctccttcgcatagccgatttcattgccgcgatgaacggcatggacgcgaagcaggacatgcaggctctgtgggacgcagaaatcgccatcatgaacggccgcgcccagacgacgatcatttcctacatcaccaaatatcgcaacgccatccgggaagccttcggtgacgaccatccgatgctgaagatcgccaccggcgatgccgcgatgtatgacgaggcccgccgggtgaagatggagaagatcgccaacaagcatggcgcgctcatcacattcgagaactaccggcaggttctgaaaatctgcgaggattgtctcaagtccagcgatcccctgatgatcggcatcggcctcatcggcatgacgggacgccgaccctatgaagtcttcacccaggcggaattttcacctgcaccctatggcaagggagtttccaaatggagcatcctgttcaacggtcaggccaagacgaaacagggcgagggcacgaaattcgggattacctatgaaattcctgtcctgacgcgctccgaaaccgtgctggctgcctataagcgcctgcgcgaaagcggacagggaaaattatggcatggcatgtcgatcgacgatttttcctcggaaacccgcctgctgctgcgcgacacggtttttaacctgttcgaggatgtctggccaaaggaagagcttcccaagccctatggcctcagacacctctatgccgaagtggcctatcacaatttcgcgccaccccatgtcaccaagaacagctatttcgccgccattcttggccacaacaataacgacctcgaaacgtcgctgtcctatatgacctatacgctgccggaagaccgcgacaatgcgctggcgcgcctgaagcggaccaatgagcggacattgcagcaaatggcgacgatcgcgcccgtgtcccgcaagggatga

SEQ ID NO: 12 - protein, 442 aa, Agrobacterium tumefaciens strain C58
  MISC_FEATURE: Protelomerase TelA
MLAAKRKTKTPVLVERIDQFVGQIKEAMKSDDASRNRKIRDLWDAEVRYHFDNGRTEKTLELYIMKYRNALKAEFGPKSTPLAICNMKKLRERLNTYIARGDYPKTGVATSIVEKIERAEFNTAGRKPTVLLRIADFIAAMNGMDAKQDMQALWDAEIAIMNGRAQTTIISYITKYRNAIREAFGDDHPMLKIATGDAAMYDEARRVKMEKIANKHGALITFENYRQVLKICEDCLKSSDPLMIGIGLIGMTGRRPYEVFTQAEFSPAPYGKGVSKWSILFNGQAKTKQGEGTKFGITYEIPVLTRSETVLAAYKRLRESGQGKLWHGMSIDDFSSETRLLLRDTVFNLFEDVWPKEELPKPYGLRHLYAEVAYHNFAPPHVTKNSYFAAILGHNNNDLETSLSYMTYTLPEDRDNALARLKRTNERTLQQMATIAPVSRKG

SEQ ID NO: 13 - DNA, 1668 bp, Vibrio parahaemolyticus phage Vp58.5 Gp40
  misc_feature: Protelomerase
atgaaactaactgacggaatggaccgcacaaagtacatcgttaaagcggccaaacatatccaagaagaaggtcaagaaaagggacctaaatacatcactgaccgctgcggtcgtgtcgctaaggatgagcacaaacgtcttggctgggttgtggaccaggtgtcaggtgagctggccagcaatccacaaatcagccataaccactatatcaatcttatgaataattaccgtagagccatcaaggccctagggtataagcatcaccaaatagaaaagacattagtaacttttatcaataaatatcaagaatatagacctgaaatagcagagatgctggacccatctttgccaattgataccttgagagagaatgtgatccttctgaaatcacaggccaggtcaaaaagtgaatttcgtagtgacctgcttggtcttcgcattgagtttcacctctactatctgtttgaaccaaagggcattgcaaccgataagcgcaaagagcaagtaaaagaagcgttgaatgaaaagcatgagaacgtcatcaagataaatggcgatcacatcaaggaactggccacaaaaattctgtcagaaaaggacccgtcatatacagaccttgcagttggccttgctcttgcgactggccgtcgagctaatgagattatgaagactgccagctttaagaaatcaggtgaacggtcgcttatgtttgagggacagctaaaaacccataaccgatacctgtttgaagaaattggagcatacgagataccttgtattgttgattcagacttagtaattaaaggattgaaattattaagaaaaaaaacaggagcggaaatcctggaatatactgatgtcactggacgtacagttaaaaaggctgttgctgacggcgacactaaggacctgagacacaatgatgcagtcaaccttcggttcactgcatcacttaaccagagagtcaaggccatactaggccatggagagtttagtttcaggacctgtcgggccatctatgtcgaaatagcattccatgagttcagacataacggagaatcgaaagcggccttccgtagcagagttcttggccactcaggtggtgataaatcaacacagaaccactatgaggggtttgagcttgattccaaggtggaaaccatcggtgtggttgatatgggccaaaacgaggctgacaagtcatacaacaagcaactgctgaagcacctggagcaatacgatgcaacaattgcagcctatctgagagcgcctaactggaaacacattcatgattggctaaaagaccaggtgaaaaacggcctgcagcttgaccaaataaccacaagctatctgagaaaaatgtgcatcatcaacaacaaaagcctcaatgcaaacaccatcgccaagtacctggaaacattgaacctagataaggttccagcagagcaagaggaaagccatcaggaagaactggagcaggaagaagatcagaaagtgtcatggccaaaagctaaagacattaaggtccagtctaaaaaagaaggtgatatgtggcatgtctggactgaggttaacggaatgcggtgggaaaattggtctaaaggtagaaaaacagaagctgtgaaggcattgcgacaacaatatgagagggaatcagcggaaatgtaa

SEQ ID NO: 14 - protein, 555 aa, Vibrio parahaemolyticus phage Vp58.5 Gp40
  MISC_FEATURE: Protelomerase
MKLTDGMDRTKYIVKAAKHIQEEGQEKGPKYITDRCGRVAKDEHKRLGWVVDQVSGELASNPQISHNHYINLMNNYRRAIKALGYKHHQIEKTLVTFINKYQEYRPEIAEMLDPSLPIDTLRENVILLKSQARSKSEFRSDLLGLRIEFHLYYLFEPKGIATDKRKEQVKEALNEKHENVIKINGDHIKELATKILSEKDPSYTDLAVGLALATGRRANEIMKTASFKKSGERSLMFEGQLKTHNRYLFEEIGAYEIPCIVDSDLVIKGLKLLRKKTGAEILEYTDVTGRTVKKAVADGDTKDLRHNDAVNLRFTASLNQRVKAILGHGEFSFRTCRAIYVEIAFHEFRHNGESKAAFRSRVLGHSGGDKSTQNHYEGFELDSKVETIGVVDMGQNEADKSYNKQLLKHLEQYDATIAAYLRAPNWKHIHDWLKDQVKNGLQLDQITTSYLRKMCIINNKSLNANTIAKYLETLNLDKVPAEQEESHQEELEQEEDQKVSWPKAKDIKVQSKKEGDMWHVWTEVNGMRWENWSKGRKTEAVKALRQQYERESAEM

SEQ ID NO: 15 - DNA, 56 bp, Escherichia coli phage N15
  misc_feature: protelomerase target sequence
tatcagcacacaattgcccattatacgcgcgtataatggactattgtgtgctgata

SEQ ID NO: 16 - DNA, 50 bp, Klebsiella phage phiK02
  misc_feature: protelomerase target sequence
cagcacacaacagcccattatacgcgcgtataatgggctattatgtgctg

SEQ ID NO: 17 - DNA, 52 bp, Yersinia enterolytica phage PY54
  misc_feature: protelomerase target sequence
tagtcacctatttcagcatactacgcgcgtagtatgctgaaataggttactg

SEQ ID NO: 18 - DNA, 90 bp, Vibrio sp. phage VP882
  misc_feature: protelomerase target sequence
gggatcccgttccatacatacatgtatccatgtggcatactatacgtatagtatgccgatgttacatatggtatcattcgggatcccgtt

SEQ ID NO: 19 - DNA, 38 bp, Borrelia burgdorferi
  misc_feature: protelomerase target sequence
tactaaataaatattatatatataattttttattagta

SEQ ID NO: 20 - DNA, 50 bp, Agrobacterium tumefaciens strain C58
  misc_feature: protelomerase target sequence
gcgatcgatcataataacaatatcatgatattgttattgtaatcgatcgc

SEQ ID NO: 21 - DNA, 56 bp, Vibrio parahaemolyticus phage Vp58.5 Gp40
  misc_feature: protelomerase target sequence
aacctgcacaggtgtacatatagtctaattagactatatgtacacctgtgcaggtt

SEQ ID NO: 22 - DNA, 26 bp, Agrobacterium tumefaciens strain C58
  misc_feature: protelomerase target sequence
aataacaatatcatgatattgttatt

SEQ ID NO: 23 - DNA, 11 bp, Artificial
  Oligonucleotide S1; Example 1
gcgtataatgg

SEQ ID NO: 24 - DNA, 71 bp, Artificial
  PEGS-1; Example 1
tatcagcacacaattgcccattatacgcgcgtataatgggcaattgtgtgctgatatgtacacttaagtag

SEQ ID NO: 25 - DNA, 45 bp, Artificial
  PEGS2; Example 1
gctatgaactaatgaccccgtaattgattactacttaagtgtaca

SEQ ID NO: 26 - DNA, 45 bp, Artificial
  PEGS3; Example 1
aagttatgtaacgcggaactccatatatgggctatgaactaatga

SEQ ID NO: 27 - DNA, 35 bp, Artificial
  PEGS4; Example 1
ccaggcgggccatttaccgtaagttatgtaacgcg

SEQ ID NO: 28 - DNA, 40 bp, Artificial
  PEGS5; Example 1
tgggcgggggtcgttgggcggtcagccaggcgggccattt

SEQ ID NO: 29 - DNA, 30 bp, Artificial
  PEGS6; Example 1
agtagatctgctagctgggcgggggtcgtt

SEQ ID NO: 30 - DNA, 74 bp, Artificial
  PEGS7; Example 1
atagtcgtgtgttaacgggtaatatgcgcgcatattacccgttaacacacgactatactagtagatctgctagc

SEQ ID NO: 31 - DNA, 79 bp, Artificial
  Oligonucleotide 1.120; Example 2
tatcagcacacaattgcccattatacgcgcgtataatggactattgtgtgctgatatgtacacttaagtagtaatcaat

SEQ ID NO: 32 - DNA, 60 bp, Artificial
  Oligonucleotide 1.112; Example 2
tgggctatgaactaatgaccccgtaattgattactacttaagtgtacatatcagcacaca

SEQ ID NO: 33 - DNA, 54 bp, Artificial
  Oligonucleotide 1.113; Example 2
ccgtaagttatgtaacgcggaactccatatatgggctatgaactaatgaccccg

SEQ ID NO: 34 - DNA, 60 bp, Artificial
  Oligonucleotide 1.114; Example 2
ctagtagatctgctagccgccaggcgggccatttaccgtaagttatgtaacgcggaactc

SEQ ID NO: 35 - DNA, 80 bp, Artificial
  Oligonucleotide 1.107v; Example2
aacctgcacaggtgtacatatagtctaattagactatatgtacacctgtgcaggttactagtagatctgctagccgccag

SEQ ID NO: 36 - DNA, 81 bp, Artificial
  Oligonucleotide 3.1
tatggaaaaacgccagcaacgcggcctttttacggttcctggccttttgctggccttttgctcacatgtagatcttgtaca

SEQ ID NO: 37 - DNA, 200 bp, Artificial
  Oligonucleotide 3.2
gggcgggggtcgttgggcggtcagccaggcgggccatttaccgtaagttatgtaacgcggaactccatatatgggctatgaactaatgaccccgtaattgattactacttaagtgtacatatcagcacacaatagtccattatacgcgcgtataatgggcaattgtgtgctgatatgtacaagatctacatgtgagcttt

SEQ ID NO: 38 - DNA, 200 bp, Artificial
  Oligonucleotide 3.3
ataatgccaggcgggccatttaccgtcattgacgtcaatagggggcgtacttggcatatgatacacttgatgtactgccaagtgggcagtttaccgtaaatactccacccattgacgtcaatggaaagtccctattggcgttactatgggaacatacgtcattattgacgtcaatgggcgggggtcgttgggcggtctcg

SEQ ID NO: 39 - DNA, 200 bp, Artificial
  Oligonucleotide 3.4
gccaaaacaaactcccattgacgtcaatggggtggagacttggaaatccccgtgagtcaaaccgctatccacgcccattgatgtactgccaaaaccgcatcaccatggtaatagcgatgactaatacgtagatgtactgccaagtaggaaagtcccataaggtcatgtactgggcataatgccaggcgggccatttaggc

SEQ ID NO: 40 - DNA, 64 bp, Artificial
  Oligonucleotide 3.5
ccattatacgcgcgtataatgggcaattgtgtgctgatagccaaaacaaactcccattgaccag

SEQ ID NO: 41 - DNA, 159 bp, Artificial
  Oligonucleotide DNA-T
tactagtcatctatcagcacacaattgcccattatacgcgcgtataatggactattgtgtgctgatatactaggcaccacctgcaggaatctactaggccgccgcaaccaaacttggatcggtgcacatgtcgaatactaggattcctgcaggtggtgc

SEQ ID NO: 42 - DNA, 159 bp, Artificial
  Oligonucleotide DNA-V
tactagtcatcaacctgcacaggtgtacatatagtctaattagactatatgtacacctgtgcaggtttactaggcaccacctgcaggaatctactaggccgccgcaaccaaacttggatcggtgcacatgtcgaatactaggattcctgcaggtggtgc

SEQ ID NO: 43 - DNA, 10 bp, Artificial
  Oligonucleotide: exemplary sequence figure 4a
tcgacgtcga